European Patent Application EP 4 800 037 A2, published September 2, 2026. Title: ANTI-CERAMIDE ANTIBODIES. Applicant: Memorial Sloan-Kettering Cancer Center. Application JP 2026-007476, filed January 20, 2026. The sequence listing filed with the application follows.

SEQUENCE LISTING (76 sequences)

SEQ ID NO: 1 - protein, 10 aa, synthetic construct
  REGION 1..10: note = HCDR1-IH
GYTFTDHTIH

SEQ ID NO: 2 - protein, 10 aa, synthetic construct
  REGION 1..10: note = HCDR1-IH-MH
GYTFTDHTMH

SEQ ID NO: 3 - protein, 17 aa, synthetic construct
  REGION 1..17: note = HCDR2-DG
YNYPRDGSTKYNEKFQG

SEQ ID NO: 4 - protein, 17 aa, synthetic construct
  REGION 1..17: note = HCDR2-DG-EG
YNYPREGSTKYNEKFQG

SEQ ID NO: 5 - protein, 17 aa, synthetic construct
  REGION 1..17: note = HCDR2-DG-DV
YNYPRDVSTKYNEKFQG

SEQ ID NO: 6 - protein, 17 aa, synthetic construct
  REGION 1..17: note = HCDR2-NE-AE
YNYPRDGSTKYAEKFQG

SEQ ID NO: 7 - protein, 11 aa, synthetic construct
  REGION 1..11: note = HCDR3
GFITTVVPSAY

SEQ ID NO: 8 - protein, 11 aa, synthetic construct
  REGION 1..11: note = LCDR1
RASKSISKYLA

SEQ ID NO: 9 - protein, 7 aa, synthetic construct
  REGION 1..7: note = LCDR2
SGSTLQS

SEQ ID NO: 10 - protein, 9 aa, synthetic construct
  REGION 1..9: note = LCDR3
QQHNEYPWT

SEQ ID NO: 11 - protein, 10 aa, Mus musculus
GYTFTDHTIH

SEQ ID NO: 12 - protein, 17 aa, Mus musculus
YNYPRDGSTKYNEKFKG

SEQ ID NO: 13 - protein, 11 aa, Mus musculus
GFITTVVPSAY

SEQ ID NO: 14 - protein, 11 aa, Mus musculus
RASKSISKYLA

SEQ ID NO: 15 - protein, 7 aa, Mus musculus
SGSTLQS

SEQ ID NO: 16 - protein, 9 aa, Mus musculus
QQHNEYPWT

SEQ ID NO: 17 - protein, 120 aa, synthetic construct
  REGION 1..120: note = Humanized VH1
QVQLVQSGAEVKKPGASVKVSCKASGYTFTDHTMHWVRQAPGQGLEWMGYNYPRDGSTKYAEKFQGRVTMTADKSTSTVYMELSSLRSEDTAVYYCAKGFITTVVPSAYWGQGTLVTVSS

SEQ ID NO: 18 - protein, 120 aa, synthetic construct
  REGION 1..120: note = Humanized VH2
QVQLVQSGAEVKKPGASVKVSCKVSGYTFTDHTIHWMRQAPGQGLEWMGYNYPRDGSTKYNEKFQGRVTMTADKSTSTVYMELSSLRSEDTAVYYCAKGFITTVVPSAYWGQGTLVTVSS

SEQ ID NO: 19 - protein, 120 aa, synthetic construct
  REGION 1..120: note = Humanized VH3
QVQLVQSGAEVKKPGATVKISCKVSGYTFTDHTIHWMQQAPGKGLEWMGYNYPRDGSTKYNEKFQGRVTITADKSTSTAYMELSSLRSEDTAVYYCAKGFITTVVPSAYWGQGTLVTVSS

SEQ ID NO: 20 - protein, 120 aa, synthetic construct
  REGION 1..120: note = Humanized VH4
QVQLVQSGAEVKKPGASVKVSCKVSGYTFTDHTIHWMRQAPGQGLEWMGYNYPREGSTKYNEKFQGRVTMTADKSTSTVYMELSSLRSEDTAVYYCAKGFITTVVPSAYWGQGTLVTVSS

SEQ ID NO: 21 - protein, 120 aa, synthetic construct
  REGION 1..120: note = Humanized VH5
QVQLVQSGAEVKKPGASVKVSCKVSGYTFTDHTIHWMRQAPGQGLEWMGYNYPRDVSTKYNEKFQGRVTMTADKSTSTVYMELSSLRSEDTAVYYCAKGFITTVVPSAYWGQGTLVTVSS

SEQ ID NO: 22 - protein, 107 aa, synthetic construct
  REGION 1..107: note = Humanized VL1
DIQLTQSPSFLSASVGDRVTITCRASKSISKYLAWYQQKPGKAPKLLIYSGSTLQSGVPSRFSGSGSGTEFTLTISSLQPEDFATYYCQQHNEYPWTFGGGTKVEIK

SEQ ID NO: 23 - protein, 107 aa, synthetic construct
  REGION 1..107: note = Humanized VL2
DVQITQSPSFLSASVGDRVTITCRASKSISKYLAWYQQKPGKANKLLIYSGSTLQSGVPSRFSGSGSGTDFTLTISSLQPEDFATYYCQQHNEYPWTFGGGTKVEIK

SEQ ID NO: 24 - protein, 107 aa, synthetic construct
  REGION 1..107: note = Humanized VL3
DVQLTQSPSSVSASVGDRVTITCRASKSISKYLAWYQQKPGKAPKLLIYSGSTLQSGVPSRFSGSGSGTDFTLTISSLQPEDFATYYCQQHNEYPWTFGPGTKVEIK

SEQ ID NO: 25 - protein, 20 aa, synthetic construct
  REGION 1..20: note = STD1 linker
NYGGGGSGGGGSGGGGSGNS

SEQ ID NO: 26 - protein, 38 aa, synthetic construct
  REGION 1..38: note = STD2 linker
NYGGGGSGGGGSGGGGSGNYGGGGSGGGGSGGGGSGNS

SEQ ID NO: 27 - skipped

SEQ ID NO: 28 - protein, 8 aa, synthetic construct
  REGION 1..8: note = H2 linker
GGGGSGNS

SEQ ID NO: 29 - protein, 10 aa, synthetic construct
  REGION 1..10: note = H3 linker
NYGGGGSGNS

SEQ ID NO: 30 - protein, 13 aa, synthetic construct
  REGION 1..13: note = H4 linker
GGGGSGGGGSGNS

SEQ ID NO: 31 - protein, 15 aa, synthetic construct
  REGION 1..15: note = H5 linker
NYGGGGSGGGGSGNS

SEQ ID NO: 32 - protein, 18 aa, synthetic construct
  REGION 1..18: note = H6 linker
GGGGSGGGGSGGGGSGNS

SEQ ID NO: 33 - protein, 8 aa, synthetic construct
  REGION 1..8: note = H7 linker
GCPPCPNS

SEQ ID NO: 34 - protein, 5 aa, synthetic construct
  REGION 1..5: note = Gly4Ser linker
GGGGS

SEQ ID NO: 35 - protein, 15 aa, synthetic construct
  REGION 1..15: note = (G4S)3 linker
GGGGSGGGGSGGGGS

SEQ ID NO: 36 - protein, 16 aa, synthetic construct
  REGION 1..16: note = H105 linker
SGGGGSGGGGSGGGGS

SEQ ID NO: 37 - protein, 20 aa, synthetic construct
  REGION 1..20: note = (G4S)4 linker
GGGGSGGGGSGGGGSGGGGS

SEQ ID NO: 38 - protein, 21 aa, synthetic construct
  REGION 1..21: note = H75 linker (NKG2A quadruple mutant)
QRHNNSSLNTGTQMAGHSPNS

SEQ ID NO: 39 - protein, 16 aa, synthetic construct
  REGION 1..16: note = H83 linker (NKG2A derived)
SSLNTGTQMAGHSPNS

SEQ ID NO: 40 - protein, 18 aa, synthetic construct
  REGION 1..18: note = H106 linker (NKG2A derived)
QRHNNSSLNTGTQMAGHS

SEQ ID NO: 41 - protein, 14 aa, synthetic construct
  REGION 1..14: note = H81 linker (NKG2D derived)
EVQIPLTESYSPNS

SEQ ID NO: 42 - protein, 20 aa, synthetic construct
  REGION 1..20: note = H91 linker (NKG2D derived)
NSLANQEVQIPLTESYSPNS

SEQ ID NO: 43 - protein, 19 aa, synthetic construct
  REGION 1..19: note = H94 linker
SGGGGSGGGGSGGGGSPNS

SEQ ID NO: 44 - protein, 19 aa, synthetic construct
  REGION 1..19: note = H111 linker
SGGGGSGGGGSGGGGSPGS

SEQ ID NO: 45 - protein, 19 aa, synthetic construct
  REGION 1..19: note = H113 linker
SGGGGSGGGGSGGGGSPAS

SEQ ID NO: 46 - protein, 18 aa, synthetic construct
  REGION 1..18: note = H114 linker
SGGGGSGGGGSGGGGSPS

SEQ ID NO: 47 - protein, 19 aa, synthetic construct
  REGION 1..19: note = H115 linker
SGGGGSGGGGSGGGGSPSS

SEQ ID NO: 48 - protein, 283 aa, synthetic construct
  REGION 1..283: note = VH2-VL1 (Lead) scFv
MEWSWVFLFFLSVTTGVHSQVQLVQSGAEVKKPGASVKVSCKVSGYTFTDHTIHWMRQAPGQGLEWMGYNYPRDGSTKYNEKFQGRVTMTADKSTSTVYMELSSLRSEDTAVYYCAKGFITTVVPSAYWGQGTLVTVSSGGGGSGGGGSGGGGSDIQLTQSPSFLSASVGDRVTITCRASKSISKYLAWYQQKPGKAPKLLIYSGSTLQSGVPSRFSGSGSGTEFTLTISSLQPEDFATYYCQQHNEYPWTFGGGTKVEIKRAAAGGGGSGGGGSHHHHHHHH

SEQ ID NO: 49 - protein, 283 aa, synthetic construct
  REGION 1..283: note = VH4-VL1 scFv
MEWSWVFLFFLSVTTGVHSQVQLVQSGAEVKKPGASVKVSCKVSGYTFTDHTIHWMRQAPGQGLEWMGYNYPREGSTKYNEKFQGRVTMTADKSTSTVYMELSSLRSEDTAVYYCAKGFITTVVPSAYWGQGTLVTVSSGGGGSGGGGSGGGGSDIQLTQSPSFLSASVGDRVTITCRASKSISKYLAWYQQKPGKAPKLLIYSGSTLQSGVPSRFSGSGSGTEFTLTISSLQPEDFATYYCQQHNEYPWTFGGGTKVEIKRAAAGGGGSGGGGSHHHHHHHH

SEQ ID NO: 50 - protein, 283 aa, synthetic construct
  REGION 1..283: note = VH5-VL1 scFv
MEWSWVFLFFLSVTTGVHSQVQLVQSGAEVKKPGASVKVSCKVSGYTFTDHTIHWMRQAPGQGLEWMGYNYPRDVSTKYNEKFQGRVTMTADKSTSTVYMELSSLRSEDTAVYYCAKGFITTVVPSAYWGQGTLVTVSSGGGGSGGGGSGGGGSDIQLTQSPSFLSASVGDRVTITCRASKSISKYLAWYQQKPGKAPKLLIYSGSTLQSGVPSRFSGSGSGTEFTLTISSLQPEDFATYYCQQHNEYPWTFGGGTKVEIKRAAAGGGGSGGGGSHHHHHHHH

SEQ ID NO: 51 - protein, 264 aa, synthetic construct
  REGION 1..264: note = VH2-VL1 scFv - no signal sequence
QVQLVQSGAEVKKPGASVKVSCKVSGYTFTDHTIHWMRQAPGQGLEWMGYNYPRDGSTKYNEKFQGRVTMTADKSTSTVYMELSSLRSEDTAVYYCAKGFITTVVPSAYWGQGTLVTVSSGGGGSGGGGSGGGGSDIQLTQSPSFLSASVGDRVTITCRASKSISKYLAWYQQKPGKAPKLLIYSGSTLQSGVPSRFSGSGSGTEFTLTISSLQPEDFATYYCQQHNEYPWTFGGGTKVEIKRAAAGGGGSGGGGSHHHHHHHH

SEQ ID NO: 52 - protein, 264 aa, synthetic construct
  REGION 1..264: note = VH4-VL1 scFv - no signal sequence
QVQLVQSGAEVKKPGASVKVSCKVSGYTFTDHTIHWMRQAPGQGLEWMGYNYPREGSTKYNEKFQGRVTMTADKSTSTVYMELSSLRSEDTAVYYCAKGFITTVVPSAYWGQGTLVTVSSGGGGSGGGGSGGGGSDIQLTQSPSFLSASVGDRVTITCRASKSISKYLAWYQQKPGKAPKLLIYSGSTLQSGVPSRFSGSGSGTEFTLTISSLQPEDFATYYCQQHNEYPWTFGGGTKVEIKRAAAGGGGSGGGGSHHHHHHHH

SEQ ID NO: 53 - protein, 264 aa, synthetic construct
  REGION 1..264: note = VH5-VL1 scFv - no signal sequence
QVQLVQSGAEVKKPGASVKVSCKVSGYTFTDHTIHWMRQAPGQGLEWMGYNYPRDVSTKYNEKFQGRVTMTADKSTSTVYMELSSLRSEDTAVYYCAKGFITTVVPSAYWGQGTLVTVSSGGGGSGGGGSGGGGSDIQLTQSPSFLSASVGDRVTITCRASKSISKYLAWYQQKPGKAPKLLIYSGSTLQSGVPSRFSGSGSGTEFTLTISSLQPEDFATYYCQQHNEYPWTFGGGTKVEIKRAAAGGGGSGGGGSHHHHHHHH

SEQ ID NO: 54 - protein, 264 aa, synthetic construct
  REGION 1..264: note = VH1-VL1 scFv
QVQLVQSGAEVKKPGASVKVSCKASGYTFTDHTMHWVRQAPGQGLEWMGYNYPRDGSTKYAEKFQGRVTMTADKSTSTVYMELSSLRSEDTAVYYCAKGFITTVVPSAYWGQGTLVTVSSGGGGSGGGGSGGGGSDIQLTQSPSFLSASVGDRVTITCRASKSISKYLAWYQQKPGKAPKLLIYSGSTLQSGVPSRFSGSGSGTEFTLTISSLQPEDFATYYCQQHNEYPWTFGGGTKVEIKRAAAGGGGSGGGGSHHHHHHHH

SEQ ID NO: 55 - protein, 264 aa, synthetic construct
  REGION 1..264: note = VH1-VL2 scFv
QVQLVQSGAEVKKPGASVKVSCKASGYTFTDHTMHWVRQAPGQGLEWMGYNYPRDGSTKYAEKFQGRVTMTADKSTSTVYMELSSLRSEDTAVYYCAKGFITTVVPSAYWGQGTLVTVSSGGGGSGGGGSGGGGSDVQITQSPSFLSASVGDRVTITCRASKSISKYLAWYQQKPGKANKLLIYSGSTLQSGVPSRFSGSGSGTDFTLTISSLQPEDFATYYCQQHNEYPWTFGGGTKVEIKRAAAGGGGSGGGGSHHHHHHHH

SEQ ID NO: 56 - protein, 264 aa, synthetic construct
  REGION 1..264: note = VH1-VL3 scFv
QVQLVQSGAEVKKPGASVKVSCKASGYTFTDHTMHWVRQAPGQGLEWMGYNYPRDGSTKYAEKFQGRVTMTADKSTSTVYMELSSLRSEDTAVYYCAKGFITTVVPSAYWGQGTLVTVSSGGGGSGGGGSGGGGSDVQLTQSPSSVSASVGDRVTITCRASKSISKYLAWYQQKPGKAPKLLIYSGSTLQSGVPSRFSGSGSGTDFTLTISSLQPEDFATYYCQQHNEYPWTFGPGTKVEIKRAAAGGGGSGGGGSHHHHHHHH

SEQ ID NO: 57 - protein, 264 aa, synthetic construct
  REGION 1..264: note = VH2-VL2 scFv
QVQLVQSGAEVKKPGASVKVSCKVSGYTFTDHTIHWMRQAPGQGLEWMGYNYPRDGSTKYNEKFQGRVTMTADKSTSTVYMELSSLRSEDTAVYYCAKGFITTVVPSAYWGQGTLVTVSSGGGGSGGGGSGGGGSDVQITQSPSFLSASVGDRVTITCRASKSISKYLAWYQQKPGKANKLLIYSGSTLQSGVPSRFSGSGSGTDFTLTISSLQPEDFATYYCQQHNEYPWTFGGGTKVEIKRAAAGGGGSGGGGSHHHHHHHH

SEQ ID NO: 58 - protein, 264 aa, synthetic construct
  REGION 1..264: note = VH2-VL3 scFv
QVQLVQSGAEVKKPGASVKVSCKVSGYTFTDHTIHWMRQAPGQGLEWMGYNYPRDGSTKYNEKFQGRVTMTADKSTSTVYMELSSLRSEDTAVYYCAKGFITTVVPSAYWGQGTLVTVSSGGGGSGGGGSGGGGSDVQLTQSPSSVSASVGDRVTITCRASKSISKYLAWYQQKPGKAPKLLIYSGSTLQSGVPSRFSGSGSGTDFTLTISSLQPEDFATYYCQQHNEYPWTFGPGTKVEIKRAAAGGGGSGGGGSHHHHHHHH

SEQ ID NO: 59 - protein, 264 aa, synthetic construct
  REGION 1..264: note = VH3-VL1 scFv
QVQLVQSGAEVKKPGATVKISCKVSGYTFTDHTIHWMQQAPGKGLEWMGYNYPRDGSTKYNEKFQGRVTITADKSTSTAYMELSSLRSEDTAVYYCAKGFITTVVPSAYWGQGTLVTVSSGGGGSGGGGSGGGGSDIQLTQSPSFLSASVGDRVTITCRASKSISKYLAWYQQKPGKAPKLLIYSGSTLQSGVPSRFSGSGSGTEFTLTISSLQPEDFATYYCQQHNEYPWTFGGGTKVEIKRAAAGGGGSGGGGSHHHHHHHH

SEQ ID NO: 60 - protein, 264 aa, synthetic construct
  REGION 1..264: note = VH3-VL2 scFv
QVQLVQSGAEVKKPGATVKISCKVSGYTFTDHTIHWMQQAPGKGLEWMGYNYPRDGSTKYNEKFQGRVTITADKSTSTAYMELSSLRSEDTAVYYCAKGFITTVVPSAYWGQGTLVTVSSGGGGSGGGGSGGGGSDVQITQSPSFLSASVGDRVTITCRASKSISKYLAWYQQKPGKANKLLIYSGSTLQSGVPSRFSGSGSGTDFTLTISSLQPEDFATYYCQQHNEYPWTFGGGTKVEIKRAAAGGGGSGGGGSHHHHHHHH

SEQ ID NO: 61 - protein, 264 aa, synthetic construct
  REGION 1..264: note = VH3-VL3 scFv
QVQLVQSGAEVKKPGATVKISCKVSGYTFTDHTIHWMQQAPGKGLEWMGYNYPRDGSTKYNEKFQGRVTITADKSTSTAYMELSSLRSEDTAVYYCAKGFITTVVPSAYWGQGTLVTVSSGGGGSGGGGSGGGGSDVQLTQSPSSVSASVGDRVTITCRASKSISKYLAWYQQKPGKAPKLLIYSGSTLQSGVPSRFSGSGSGTDFTLTISSLQPEDFATYYCQQHNEYPWTFGPGTKVEIKRAAAGGGGSGGGGSHHHHHHHH

SEQ ID NO: 62 - protein, 271 aa, synthetic construct
  REGION 1..271: note = Mouse 6B5 scFv
MKKTAIAIAVALAGFATVAQAQVQLQQSDAELVKPGASVKISCKVSGYTFTDHTIHWMKQRPEQGLEWIGYNYPRDGSTKYNEKFKGKATLTADKSSSTAYMQLNSLTSEDSAVYFCAKGFITTVVPSAYWGQGTLVTVSAGGGGSGGGGSGGGGSDVQITQSPSYLAASPGETITINCRASKSISKYLAWYQEKPGKTNKLLIYSGSTLQSGIPSRFSGSGSGTDFTLTISSLEPEDFAMYYCQQHNEYPWTFGGGTKLEIKGSHHHHHH

SEQ ID NO: 63 - protein, 120 aa, synthetic construct
  REGION 1..120: note = Murine 6B5 VH parental
QVQLQQSDAELVKPGASVKISCKVSGYTFTDHTIHWMKQRPEQGLEWIGYNYPRDGSTKYNEKFKGKATLTADKSSSTAYMQLNSLTSEDSAVYFCAKGFITTVVPSAYWGQGTLVTVSA

SEQ ID NO: 64 - protein, 107 aa, synthetic construct
  REGION 1..107: note = Murine 6B5 VL parental
DVQITQSPSYLAASPGETITINCRASKSISKYLAWYQEKPGKTNKLLIYSGSTLQSGIPSRFSGSGSGTDFTLTISSLEPEDFAMYYCQQHNEYPWTFGGGTKLEIK

SEQ ID NO: 65 - DNA, 861 bp, synthetic construct
  misc_feature 1..861: note = VH3-VL3 scFv nucleic acid sequence
  source 1..861: mol_type = other DNA
atgaagtaccttcttcccaccgccgcggctgggttgttgttacttgcagcacaaccggcgatggctcaagtccagttagttcagtcgggggccgaagtaaagaagccaggtgctactgtgaaaatttcgtgcaaagtgagcggatacacattcacggaccacacgattcactggatgcagcaagctccgggcaagggtcttgagtggatgggctacaactatccgcgtgacggatcaacaaaatacaatgaaaaatttcaagggcgtgttacaattaccgcggataaatccacgagtactgcctacatggagttgtcctcacttcgttcagaggacacagcagtgtactattgtgctaaagggttcatcacgaccgtggtcccctctgcttattggggccaaggaacacttgtgactgtgtcttctgggggcggggggagcggaggcggaggtagcggtggcgggggtagtgacgttcaactgactcaatcgccttcatccgttagcgccagcgtaggcgaccgtgtgaccatcacgtgccgcgcgtccaaaagtatcagcaagtacctggcctggtaccaacaaaaacccggaaaggcaccgaagttgttgatttattccggttcaacattacaaagcggcgttccgagtcgtttcagtggtagcggttccggcacagattttaccttgaccatttcctccctgcagccagaagactttgctacttattactgtcaacagcacaatgagtacccgtggacgtttgggcctggaactaaggttgagattaagcgtgctgctgccgggggcggtggttccggaggaggaggaagtcaccaccaccatcaccatcatcatggt

SEQ ID NO: 66 - DNA, 861 bp, synthetic construct
  misc_feature 1..861: note = VH3-VL2 scFv nucleic acid sequence
  source 1..861: mol_type = other DNA
atgaaatatctgctgccaactgcggcagcaggtctgttgcttctggccgctcaaccggccatggctcaagtccagttagttcagagtggggcagaggttaaaaaaccgggagctacagtaaagatcagctgtaaagtatcaggttatacatttactgaccatactatccactggatgcaacaggcgccagggaaaggtttggagtggatgggatataattatccacgcgacgggtcaactaagtacaacgagaagtttcaaggccgtgtaacgattaccgcggacaaaagcacgagtacagcgtacatggaattatcatctttgcgctcggaggacacagcggtctattactgtgccaagggtttcatcactactgtggtaccaagtgcgtattggggtcaaggaacccttgttacggtgtcatcagggggtggcggaagtggcggtggtggatcgggcggaggtggaagcgatgttcagatcacacagtcgccctcgttcctgagtgcaagtgtcggtgatcgtgtgactattacgtgtcgtgcatcgaaatcaatctcaaagtatctggcttggtaccagcaaaaacctggaaaggctaacaaattgttgatctattccgggagcacccttcaaagcggtgtcccctctcgtttctccggatccgggtcagggaccgactttactctgactatttccagtcttcagccggaagattttgcgacttactattgccagcagcataatgagtacccatggacttttggcggtggcacaaaggtcgagattaagcgtgcagctgccggtggtggaggttcgggtgggggcggttctcatcatcaccatcatcaccatcatggt

SEQ ID NO: 67 - DNA, 861 bp, synthetic construct
  misc_feature 1..861: note = VH3-VL1 scFv nucleic acid sequence
  source 1..861: mol_type = other DNA
atgaaatatttgcttccgactgccgccgcaggtctgttacttttagcagcgcagcccgctatggcacaggtccagttagttcaatcaggagcggaggtgaagaagccgggagccacggttaaaatctcatgcaaggtgtccggctatacatttaccgaccacacgattcactggatgcagcaagctcccgggaaggggcttgaatggatggggtacaattatccacgcgatggttccaccaagtataacgaaaaatttcaaggtcgtgtcaccattaccgctgacaaaagcacgtctacagcgtacatggagctgagtagcttgcgctcagaggacacagccgtatactattgcgcaaaaggtttcatcacgaccgtagtcccctctgcgtattggggacaggggaccctggtcacggtctcctccgggggcggaggatcgggaggcggggggtctggaggtggtggatctgacatccagcttacccaatcgcctagcttcttgagtgctagtgtaggcgaccgtgttactatcacttgtcgcgcttctaagagcattagcaaatacttagcctggtaccaacaaaagccgggaaaggcacccaagctgttaatttatagtgggtctacccttcagtccggcgtaccctcacgcttttccggcagtggctcgggtaccgaatttacccttacgatttcttcgcttcaacccgaagattttgcaacgtactactgtcagcagcacaacgagtatccctggacattcggcggagggacaaaagtagaaatcaagcgtgcagccgcaggtggcggcgggtctggcggcggagggagtcaccatcaccatcatcatcatcatgga

SEQ ID NO: 68 - DNA, 861 bp, synthetic construct
  misc_feature 1..861: note = VH2-VL3 scFv nucleic acid sequence
  source 1..861: mol_type = other DNA
atgaaatatttgttacctaccgctgcggcaggacttctgcttttggccgctcagcccgcaatggctcaagtgcaattggttcagtcaggggccgaagtaaaaaagccaggcgcgagcgtaaaagtgagttgcaaggtctccggttacacgtttaccgatcacacgattcactggatgcgtcaagctccaggccagggtcttgaatggatgggttacaactatcctcgcgatggttcgaccaagtataacgagaagtttcagggccgtgtcacaatgaccgccgacaaatcaacgagcactgtctacatggagctgtcatccctgcgcagcgaggatacagctgtgtactactgtgccaagggcttcattactaccgtcgtccccagcgcgtactggggtcaaggtacactggtaacagtttcatccggaggagggggaagcggcggcggtggatctggcggcggtgggtcagacgttcaacttacccagtcgccttcttccgtgagtgcctctgtcggggatcgtgttaccatcacttgccgcgcatctaagtcaatttctaaatatttggcctggtatcagcagaaacccggtaaagcgcccaaattgttgatctattccggcagtaccttgcaatccggggtgccttcgcgcttctcggggagtggaagcggcacggatttcactttaacgatctcgagtttgcagccggaagattttgcgacttactattgtcagcagcataacgaatatccatggacctttggccctggtacgaaagtagaaatcaaacgtgcagcagccggtgggggtggctccggtggcggtgggtcgcatcaccaccaccatcatcatcacggt

SEQ ID NO: 69 - DNA, 861 bp, synthetic construct
  misc_feature 1..861: note = VH2-VL2 scFv nucleic acid sequence
  source 1..861: mol_type = other DNA
atgaagtacctgttgcccacagccgctgctgggttactgcttcttgctgcccagcccgcaatggcgcaagtgcaattagtccagtctggagcagaggttaaaaagccgggagcttcagtgaaggtctcctgtaaggtaagtggttatacattcaccgatcacacaatccattggatgcgccaggccccaggtcagggtcttgaatggatgggctataactacccgcgtgatggctcaactaagtataacgagaagtttcaggggcgcgttacaatgactgcggataaaagcacgtcgacggtgtacatggaattgtcaagccttcgttccgaagataccgcagtttactattgtgctaagggctttatcactaccgtggtacccagtgcgtactgggggcagggaaccctggtaaccgtgtcatcgggcggaggcggaagcgggggaggtggcagtggaggtggcgggtctgacgttcaaatcacccagtcaccgtcatttctttccgcgtctgtgggtgaccgcgtaacaattacttgccgtgcttcgaaaagcatttcgaaataccttgcctggtaccaacagaaaccggggaaagcaaacaaacttttaatctacagcgggagcacgcttcaatccggcgtcccatcccgtttttctggctccggcagcgggaccgacttcaccttaactatttcttcccttcaaccggaggactttgcgacgtattactgtcaacaacacaatgagtatccgtggactttcggaggcggaactaaggttgaaatcaagcgtgctgctgctggcgggggaggctcaggcggagggggatcacatcatcatcaccatcatcatcacgga

SEQ ID NO: 70 - DNA, 861 bp, synthetic construct
  misc_feature 1..861: note = VH2-VL1 scFv nucleic acid sequence
  source 1..861: mol_type = other DNA
atgaaatacttgctgccgactgccgcagcgggattattattacttgcggctcagccggctatggcgcaggtccagttagttcagagtggggcagaagtgaagaaacccggtgcatctgtaaaggtctcatgtaaagtatctggctacaccttcactgaccacactatccactggatgcgtcaagcaccaggacaaggtttagagtggatgggatataactatccgcgtgacgggagtacgaagtataacgaaaaatttcagggccgtgtaaccatgaccgcggataaatccacttccactgtctatatggaattatcgtcgttacgtagcgaggacacggcggtatattattgcgccaaagggtttatcacgactgttgtgccgtccgcttactgggggcaagggactttagtgaccgtgtccagcggaggggggggtagcgggggtggcgggagtggtggtgggggttcggacattcagcttacccaatcccctagctttttgtcagcctccgttggcgatcgtgtaactattacgtgccgcgcctccaagtccatttcaaaatatttagcctggtaccaacagaagccaggaaaagctcctaaattactgatttactcaggttccacattgcagtcgggcgtaccaagccgtttttcgggaagtggtagcgggaccgagtttacattgacgattagtagtcttcaaccggaggattttgcaacctactattgtcagcagcacaacgagtacccatggacctttggaggcggtaccaaagtggaaattaaacgcgcagcagcaggcggcggtggttcagggggaggaggctcgcatcaccaccatcatcatcaccacggt

SEQ ID NO: 71 - DNA, 861 bp, synthetic construct
  misc_feature 1..861: note = VH1-VL3 scFv nucleic acid sequence
  source 1..861: mol_type = other DNA
atgaaataccttttgccgactgccgccgcaggattattgttactggcggctcagccggctatggcccaagtccaattagttcaatcaggggcagaagttaagaagcccggagcaagtgtcaaggtctcatgcaaagcctccggttacacctttaccgaccacacgatgcactgggttcgccaagctcccggacagggcctggaatggatgggttataattatccgcgtgatggtagcacgaaatacgcggaaaaattccaaggtcgcgttacgatgaccgcggacaagtctactagcaccgtgtacatggaacttagctcgctgcgttcggaagatacggcggtgtactactgtgcgaaaggtttcatcactacagtagtgccaagtgcgtattggggtcaaggcacgctggtaacggtttcaagtggtggcggcggtagcggcggcggcggcagcggaggagggggatcggatgtccaacttacgcaatctccgtcctctgtttccgcaagtgtgggcgaccgcgtaaccatcacttgccgtgctagtaaaagcatttctaagtatttagcgtggtatcaacagaagcccggaaaggcgccaaagctgttgatttattccgggagtacattacaatctggcgtgccgtcccgcttctccggcagcggtagtggtactgacttcacgctgacaattagttcacttcagccagaggattttgcgacatattattgccagcagcataacgaatacccatggaccttcggtcctggaaccaaggttgaaatcaaacgtgctgcggccggcggcggtgggagcggagggggcgggtcacatcatcatcatcatcaccatcatggt

SEQ ID NO: 72 - DNA, 861 bp, synthetic construct
  misc_feature 1..861: note = VH1-VL2 scFv nucleic acid sequence
  source 1..861: mol_type = other DNA
atgaaataccttcttcccaccgcagcagcgggattgttattattggctgcacaacctgcgatggctcaagtacagttggtgcagtcaggggcggaagtcaagaaaccaggcgcttcagtgaaagtttcgtgtaaagcatccggctatacttttaccgaccacaccatgcactgggttcgccaagctcctggacagggtctggaatggatggggtacaactatccccgcgatggatccacaaagtacgcggagaagttccaaggacgtgtaacaatgacggccgataaaagcacttccacagtctatatggaactttcgtctcttcgttctgaggacacagcagtttactactgtgctaaaggatttatcactaccgtcgttccgtctgcatattgggggcagggcacgttagtaacagtcagctccgggggcgggggctcagggggcggtggatcagggggaggcggctctgacgtgcagatcactcagtcgcctagctttctttcggctagtgtcggggatcgcgtcactatcacatgccgcgccagcaaaagcatctctaaatacctggcttggtaccaacaaaaacccggaaaggctaataagttgctgatctacagtgggagtactttgcagtcgggggtgccgagtcgtttttcaggtagcgggtcgggcacggactttacccttacaatttcctccctgcagcccgaggactttgccacatattattgtcaacagcacaacgagtacccgtggacgtttgggggaggtaccaaagtggaaatcaagcgtgcagcggccgggggaggtggaagcggcggcggtggaagtcaccatcatcaccaccaccatcacgga

SEQ ID NO: 73 - DNA, 861 bp, synthetic construct
  misc_feature 1..861: note = VH1-VL1 scFv nucleic acid sequence
  source 1..861: mol_type = other DNA
atgaaatacctgttacctactgctgccgcaggtttgttgcttctggcggctcaaccggccatggcacaggttcagctggtgcaatcaggcgccgaagtcaaaaaaccgggtgcaagcgtcaaggtgagctgtaaggcaagcggatatacttttacagatcatacaatgcactgggtacgccaggcaccaggccagggccttgaatggatgggatataactacccacgtgatggatctactaaatatgccgagaagttccagggtcgcgttaccatgactgctgataaaagtacatcaactgtatacatggaacttagctcattgcgttccgaagatactgccgtgtactattgtgcaaaggggtttatcacgacagtcgttccatcggcatattggggccagggaacgttagtaacagtcagcagtgggggtggggggtcaggcggaggagggtctggtggggggggttctgacatccagttgacacagtccccatcctttttgtctgcatcggttggggaccgcgtgacgattacttgtcgcgcgtccaagtctatcagcaaatatttagcatggtatcaacaaaaacctggcaaggctcccaagttacttatttactccggtagtactcttcagtcgggagtgccttcccgttttagcgggtctggttcaggcacggagtttacccttacaattagttctctgcagcccgaggattttgcaacttactactgccagcaacacaatgagtacccctggacattcggcggtgggacaaaagtcgagattaagcgtgccgctgccggtggaggagggtcagggggtggcggcagtcatcaccaccatcaccatcatcatgga

SEQ ID NO: 74 - DNA, 861 bp, synthetic construct
  misc_feature 1..861: note = 6B5 scFv nucleic acid sequence
  source 1..861: mol_type = other DNA
atgaagtacttattgcccactgctgctgctggattattattgttggcagcgcaaccggccatggcgcaggtccaacttcagcagtcagatgccgaacttgtaaagccgggtgcaagcgtgaaaatctcatgtaaagtatctggttatacgtttacagatcacaccatccactggatgaagcaacgccctgagcagggtttagagtggattggctataattatccgcgcgacggttcgacaaaatacaacgaaaagttcaagggcaaggcaacgcttaccgccgataagagttcaagtacagcatatatgcaactgaacagcttaactagcgaagatagcgcagtttacttttgcgcgaagggatttatcaccaccgtggttccgagtgcctactggggacagggcacattggttacagtcagtgcaggaggaggagggtccggtggcggaggatcgggtgggggtggatcagatgtccaaatcacacaatcgccatcctacttggccgcctcgcccggagaaaccatcactattaattgccgcgcgagcaagtctatttccaagtatttggcatggtaccaagaaaagcccggtaaaactaacaaacttttgatctactctgggtccacgctgcagtcaggaatcccatcccgtttctcgggcagcggatctgggacagacttcacgttgacaatttcgagccttgagccggaagatttcgcaatgtactactgtcagcaacataacgagtacccttggacatttggcgggggcacaaagcttgaaattaaacgcgctgctgccggaggaggtggttcggggggagggggttctcatcatcaccaccatcaccaccacgga

SEQ ID NO: 75 - protein, 19 aa, synthetic construct
  REGION 1..19: note = Signal sequence
MEWSWVFLFFLSVTTGVHS

SEQ ID NO: 76 - protein, 22 aa, synthetic construct
  REGION 1..22: note = C-terminal tag
RAAAGGGGSGGGGSHHHHHHHH